European Patent Application EP 4 356 917 A1, published April 24, 2024. Title: Use for combination therapy in preventing and treating metabolic disease of Lactobacillus fermentum strain and natural killer cells. Applicant: GI Cell, Inc. The sequence listing filed with the application follows.

SEQUENCE LISTING (1 sequence)

SEQ ID NO: 1 - DNA, 1441 bp, Artificial Sequence
  GB102_16S_full
gcaagtcgaacgcgttggcccaattgattgatggtgcttgcacctgattgattttggtcgccaacgagtggcggacgggtgagtaacacgtaggtaacctgcccagaagcgggggacaacatttggaaacagatgctaataccgcataacaacgttgttcgcatgaacaacgcttaaaagatggcttctcgctatcacttctggatggacctgcggtgcattagcttgttggtggggtaatggcctaccaaggcgatgatgcatagccgagttgagagactgatcggccacaatgggactgagacacggcccatactcctacgggaggcagcagtagggaatcttccacaatgggcgcaagcctgatggagcaacaccgcgtgagtgaagaagggtttcggctcgtaaagctctgttgttaaagaagaacacgtatgagagtaactgttcatacgttgacggtatttaaccagaaagtcacggctaactacgtgccagcagccgcggtaatacgtaggtggcaagcgttatccggatttattgggcgtaaagagagtgcaggcggttttctaagtctgatgtgaaagccttcggcttaaccggagaagtgcatcggaaactggataacttgagtgcagaagagggtagtggaactccatgtgtagcggtggaatgcgtagatatatggaagaacaccagtggcgaaggcggctacctggtctgcaactgacgctgagactcgaaagcatgggtagcgaacaggattagataccctggtagtccatgccgtaaacgatgagtgctaggtgttggagggtttccgcccttcagtgccggagctaacgcattaagcactccgcctggggagtacgaccgcaaggttgaaactcaaaggaattgacgggggcccgcacaagcggtggagcatgtggtttaattcgaagctacgcgaagaaccttaccaggtcttgacatcttgcgccaaccctagagatagggcgtttccttcgggaacgcaatgacaggtggtgcatggtcgtcgtcagctcgtgtcgtgagatgttgggttaagtcccgcaacgagcgcaacccttgttactagttgccagcattaagttgggcactctagtgagactgccggtgacaaaccggaggaaggtggggacgacgtcagatcatcatgccccttatgacctgggctacacacgtgctacaatggacggtacaacgagtcgcgaactcgcgagggcaagcaaatctcttaaaaccgttctcagttcggactgcaggctgcaactcgcctgcacgaagtcggaatcgctagtaatcgcggatcagcatgccgcggtgaatacgttcccgggccttgtacacaccgcccgtcacaccatgagagtttgtaacacccaaagtcggtggggtaaccttttaggagccagcc